European Patent Specification EP 2 878 192 B1, published December 3, 2025. Title: Disease Resistance Loci in Onion. Applicant: Seminis Vegetable Seeds, Inc. The sequence listing filed with the application follows.

SEQUENCE LISTING (240 sequences)

SEQ ID NO: 1 - DNA, 121 bp, Artificial sequence
  Marker sequence
  misc_feature (69)..(69): n is a, c, g, or t
  misc_feature (93)..(93): n is a, c, g, or t
  misc_feature (119)..(119): n is a, c, g, or t
aaggtttgtaaccaaactctgaccttagatgttatgattgtgtgcacaagctctactcttscagcaaangatagcaatttggatctccaaccntccaacttctctctaatatatatatnaa

SEQ ID NO: 2 - DNA, 121 bp, Artificial sequence
  Marker sequence
gccttctcttcgatttttcattgacgaaggtgatgatgctttgccgaatgatccaatgctyttccatactaaaagaacctaccagcctagcactatcaaacgcaagaggactcatggttat

SEQ ID NO: 3 - DNA, 121 bp, Artificial sequence
  Marker sequence
  misc_feature (34)..(34): n is a, c, g, or t
gcggaaggtcgcgatcctcggggccgctgggggnattgggcagcctttgtcacttctgatraagcttaatcctcttgttaccaagctagctctttatgatattgctggtactcctggcgtg

SEQ ID NO: 4 - DNA, 121 bp, Artificial sequence
  Marker sequence
tttcttgacattggacgatgcgatcaagactacaaataggagggttaatgccttggagagygttgtcaaaccaaggttggagaataccattacctatatcaagggagagctggatgagttg

SEQ ID NO: 5 - DNA, 121 bp, Artificial sequence
  Marker sequence
  misc_feature (107)..(107): n is a, c, g, or t
ctcaaaaccaccaccggtcgcattaagcaatgctagagaaagtattctgttaggtgcaatygctgccaacttgcaagcaatcattgctcccatggagtgaccaaaancatgagctttagtc

SEQ ID NO: 6 - DNA, 121 bp, Artificial sequence
  Marker sequence
ttcccaagagattatgtaccgtggtcctctagctcttttcggtgtagggcttgatgattayttcccaatgattaatatatattattaattaactcagactttgactgcactatagtgtcac

SEQ ID NO: 7 - DNA, 121 bp, Artificial sequence
  Marker sequence
  misc_feature (88)..(88): n is a, c, g, or t
atcaaataacttgatggtttctgaggaatcccatgatgtcaaatccgttttattagctaamgcaaatgaccagtgcaatttagccatntcaaaatgttgctgtccaagtgcaagtaaccct

SEQ ID NO: 8 - DNA, 121 bp, Artificial sequence
  Marker sequence
tgaatcagaaggttctctttgtgcaatttgtatccctggcatactataatatacgaaatgwaatcatctcttataacctggtaggacataggtagaaaatctaactggatgattagccaat

SEQ ID NO: 9 - DNA, 121 bp, Artificial sequence
  Marker sequence
  misc_feature (86)..(86): n is a, c, g, or t
  misc_feature (102)..(102): n is a, c, g, or t
gcttgaaaacatagttaagcaactttttcctcaagctggttgtcaatcttggtcacctagratggtacagccgatttggaaaacantatgggaaactaaaantgcacaattgagagaaggt

SEQ ID NO: 10 - DNA, 121 bp, Artificial sequence
  Marker sequence
ttccattgcttctctgcctttgatctccttccatttcttcagccctactttgtcacgattstcaaagctagggttagttttacttttgaattcgattttgaattcttaattcttatgattt

SEQ ID NO: 11 - DNA, 121 bp, Artificial sequence
  Marker sequence
  misc_feature (13)..(13): n is a, c, g, or t
tctggattgaaanttaatggcagcaaggttgagaaagctgaagagaaggtggaaaagatgyctgctttgacgctgaaaccagagaaggttaaagatgcatcgaaggctgaggctgttgtca

SEQ ID NO: 12 - DNA, 121 bp, Artificial sequence
  Marker sequence
  misc_feature (105)..(106): n is a, c, g, or t
aatgacagtaaaatggaaaattgttcaggtttgagcctgcggcatcatgccctccaaatayggagtccattttaacaatccttatttagaattactttggtaaannaagcagagagattaa

SEQ ID NO: 13 - DNA, 121 bp, Artificial sequence
  Marker sequence
tttggaatttataataggtagtgaaaagaaatgtctgaattcagagctctggcatgcatgygctggacctcttgtatgtttgccaacaatcgggactcgagtagtttacttccctcaaggc

SEQ ID NO: 14 - DNA, 121 bp, Artificial sequence
  Marker sequence
  misc_feature (9)..(9): n is a, c, g, or t
  misc_feature (15)..(15): n is a, c, g, or t
  misc_feature (94)..(94): n is a, c, g, or t
ttcatgcangcatanattgatgtatgttgtatgtaaacaataacagtaagttttgtgttgytattgtaggtggagggagaatgcgaaagaagcngttgaagaactgggagttgctttgaaa

SEQ ID NO: 15 - DNA, 121 bp, Artificial sequence
  Marker sequence
  misc_feature (91)..(91): n is a, c, g, or t
caatcccacctacacacacatttccacacgttgcattttgtgagtttatatactttctgtygttatcttcatagtcaaccttgcttatttnaacaataatataaaagtgcttttggtaaaa

SEQ ID NO: 16 - DNA, 121 bp, Artificial sequence
  Marker sequence
tctttcgaatgtgtattctgaagtgaacagatgggatgatgcagagacgacgaggattagyatgaagaattgtaatgtagataaattgcctggatggagttgtatagaggttaatggaaag

SEQ ID NO: 17 - DNA, 121 bp, Artificial sequence
  Marker sequence
  misc_feature (5)..(5): n is a, c, g, or t
  misc_feature (104)..(104): n is a, c, g, or t
  misc_feature (115)..(115): n is a, c, g, or t
caaancatagccaacctctgccagtaagttcaactaccctccaagcactacctttcacctrcactacagctacttcaccttcttctaccttctgcccgcaaatnccatcactacnccaacc

SEQ ID NO: 18 - DNA, 121 bp, Artificial sequence
  Marker sequence
ggcttatgaccaggcagcttttgccatgagggggtcgctggcaattttgaacttctcagtsgaaacagttgttgaatctttgagagaagtcaagtgcctaaaagctggaggagagtcccct

SEQ ID NO: 19 - DNA, 121 bp, Artificial sequence
  Marker sequence
  misc_feature (11)..(11): n is a, c, g, or t
  misc_feature (95)..(95): n is a, c, g, or t
gcttcagaaanccttaagttttatttcttctgcatcatcaccccctcttccctatagttcsgattactatattcccgccgtacaatttccgaaancacctccaaatcttaccgtttctcaa

SEQ ID NO: 20 - DNA, 121 bp, Artificial sequence
  Marker sequence
  misc_feature (34)..(34): n is a, c, g, or t
ggcttatgaccaggcagcttttgccatgaggggntcgctggcaattttgaacttctcagtsgaaacagttgttgaatctttgagagaagtcaagtgcctaaaagctggaggagagtcccct

SEQ ID NO: 21 - DNA, 121 bp, Artificial sequence
  Marker sequence
  misc_feature (6)..(6): n is a, c, g, or t
agaaangaagaagaaaaacaatcgaatcccctacctcttatcagaacatcgacccgaaccscacaaaccacccaatattccattgcctcatcaaaaattgcctcgccgccttcacccagaa

SEQ ID NO: 22 - DNA, 121 bp, Artificial sequence
  Marker sequence
  misc_feature (9)..(9): n is a, c, g, or t
aattaaaantaaatggatcacagacattagtatgaaagcaagcaatatataattagaattyagggctgttttgctagaaatttgagttttgcatcttgcattttcaatatgcatgttaaaa

SEQ ID NO: 23 - DNA, 121 bp, Artificial sequence
  Marker sequence
  misc_feature (12)..(12): n is a, c, g, or t
cctaaccatggnatttgtccagctaagatccccttcaagagcaagattctcaatatttagyattagcggtttcccaaactacactcaagatcagggcaggccctgtatactgggttgctct

SEQ ID NO: 24 - DNA, 121 bp, Artificial sequence
  Marker sequence
ttaataaactgaaaaggaggattcattcattcatgttaaagtgcataaaataatagatgaygatgacgatgatgatttggttttcgattttcttacccttgcaaaagctcgagaagctgtg

SEQ ID NO: 25 - DNA, 121 bp, Artificial sequence
  Marker sequence
  misc_feature (4)..(4): n is a, c, g, or t
  misc_feature (19)..(19): n is a, c, g, or t
aaangagaagagaaaaaancatgccccttatcttgctatttatctcatttaatctcttaaytactgcatccgcatctgatgcagaggaatcccttcttaactggagatcgtctcttataaa

SEQ ID NO: 26 - DNA, 121 bp, Artificial sequence
  Marker sequence
atttcgttctaaggatggggagtggcactgttatgtggataatgctgtctggtactatgcyatgttattagttggtgacagttatattatcatacactacaaaaattgcatgggttaattg

SEQ ID NO: 27 - DNA, 121 bp, Artificial sequence
  Marker sequence
aattcctcggagatggatattcttctctgtaaatagcctcgagattaaatggcctaaatcraaacccattaacatatgatatccaacaaacaaagtaggacccacagatggaattccttca

SEQ ID NO: 28 - DNA, 315 bp, Artificial sequence
  Marker sequence
gtattcaagttggcccacgtttcctcaactttatattgatggggagttttatggagggtgtgatattactgttgaagcataccagagtggggaactgcaggaagcaatagaaaaagcaatgtgttcttaataatgtctcagttatarccttctatgctccattcatgcaaagttacacttatttattaattatgttattatataatatatatctgcaattttcatatttcagatctgtggatgacacttaccatttagttgcttctggtgtttatatttattctacaaagaccatttactgagttttcaaatgct

SEQ ID NO: 29 - DNA, 121 bp, Artificial sequence
  Marker sequence
  misc_feature (23)..(23): n is a, c, g, or t
  misc_feature (99)..(99): n is a, c, g, or t
  misc_feature (104)..(104): n is a, c, g, or t
  misc_feature (114)..(114): n is a, c, g, or t
catcttataagtaatatactttnaacttttaaggatcttcaaatattctcttataaattaraggccccaagattaatccaaactgaattcataaacaantaaantatctatttnagtttct

SEQ ID NO: 30 - DNA, 121 bp, Artificial sequence
  Marker sequence
  misc_feature (58)..(58): n is a, c, g, or t
aagctgtgatttgtgcacactggtgtgcaggtgcactgtggatagtagcagttgtttnatygggtgatggctagtttggactgtggtcattaatgtttagaggctaaagcagctggttgaa

SEQ ID NO: 31 - DNA, 121 bp, Artificial sequence
  Marker sequence
  misc_feature (7)..(7): n is a, c, g, or t
  misc_feature (33)..(33): n is a, c, g, or t
  misc_feature (97)..(97): n is a, c, g, or t
aaattanttactgtaaattcatcaaaccctaantcaatcatgcaagtgtgcaattacaccrctcaagtcccaccatcatacaatacttatcgatttngatgactttcaaagtttagtgcta

SEQ ID NO: 32 - DNA, 121 bp, Artificial sequence
  Marker sequence
tttgaagcggaaagatatgtctgttgtggtgtcaatgcgcataataaagaaagcatcaaakgggtaactactatttcaaaattcatgtattcaatcatattgtttatgggctttcgtcgtg

SEQ ID NO: 33 - DNA, 121 bp, Artificial sequence
  Marker sequence
  misc_feature (21)..(21): n is a, c, g, or t
  misc_feature (106)..(106): n is a, c, g, or t
ttactattaatatcatccatntaaactgttacgtcatttcgaaattttcatctcactaaamggtgcaaattgatatgatccatcgaaaatatttatttaaccatcnatttcaaacgtagtt

SEQ ID NO: 34 - DNA, 121 bp, Artificial sequence
  Marker sequence
  misc_feature (16)..(16): n is a, c, g, or t
ttgtcctaacccctanatcatatagtatctgtgctccaatgccatattctcgtgaatcaayaggtaaccccaaatcttcgttggcttccacagtgtcacggccagcatcttgcagattata

SEQ ID NO: 35 - DNA, 121 bp, Artificial sequence
  Marker sequence
cactaaaggatctgagcaaacagctgtagaagttaatgatagtgaaagtgatttgaaccgracaattttcataaacaatattccatttgatgctgacagtgaagaggtgaaaaagagattc

SEQ ID NO: 36 - DNA, 121 bp, Artificial sequence
  Marker sequence
  misc_feature (16)..(16): n is a, c, g, or t
tgcagatccaagtaantatggtatttttaaattgatagctatcgattattttggacctttyctcttttctgcatttgatgattgcaaatgtgttctgatattattatttttcatattttta

SEQ ID NO: 37 - DNA, 121 bp, Artificial sequence
  Marker sequence
  misc_feature (86)..(86): n is a, c, g, or t
tttgatgcgcctaggaccccaacttaaagaaagccactttgaacgtgagaatgattctgcrtatagttcatcatttagcatccccnttcacaaataatgcaaaacttcattctcagattgc

SEQ ID NO: 38 - DNA, 121 bp, Artificial sequence
  Marker sequence
cgcttggcatcagtacagtagttgtaaatcatgaacttcctctgcacccacctcattctcytgtaactcaccgaatccaactcgtggttataccaatctgctggcgaagccgttgacaaca

SEQ ID NO: 39 - DNA, 121 bp, Artificial sequence
  Marker sequence
  misc_feature (2)..(2): n is a, c, g, or t
  misc_feature (60)..(60): n is a, c, g, or t
anttaagggagtttgtgtaaatatcaacaaggatacgtagtccatcactactgtcatggnrgttagacgctccggctttggtcagtgaagttacaggttgaatcatggtagtgtcattcaa

SEQ ID NO: 40 - DNA, 121 bp, Artificial sequence
  Marker sequence
ataaattgggatcagccagaaaatgctgaaacacacctatcaacaatttataccagaatcrctatttacagccaacatgctagaggcacttcaataaaatgtttagacagatcagtcattt

SEQ ID NO: 41 - DNA, 121 bp, Artificial sequence
  Marker sequence
aagaattcacttgttgatagcttcattgtcttgctggttttcaactaatctcatattctargttgccctgaaattaaatgtaaatgggaaaaatgtgaaaaggcaggttagaatcttatac

SEQ ID NO: 42 - DNA, 121 bp, Artificial sequence
  Marker sequence
ctcaataggctttcttggtgaggcagagtaatcggcatgtcttcttggtgaagcagagtgrtcagtttgccttcttggtgcaggagagtacgaccttgatgtatggcgagctcttgaagat

SEQ ID NO: 43 - DNA, 121 bp, Artificial sequence
  Marker sequence
  misc_feature (10)..(10): n is a, c, g, or t
taggtaaaanttaaagagaaaagcatcgtaaataattaagtcacaaagcagcaggtgtgtmgagtctacactaaaccaatcctttaagaagtgtaccacttatatacgattaaatgtatta

SEQ ID NO: 44 - DNA, 121 bp, Artificial sequence
  Marker sequence
cctaatttttctcctcaaatatcccatttgtttctaactaaatctcaaaggaaaagctttyattgcacgataacggttaatttaatcattcttcaagctacacaatcagtcaatcagtcgt

SEQ ID NO: 45 - DNA, 121 bp, Artificial sequence
  Marker sequence
  misc_feature (34)..(34): n is a, c, g, or t
aatttcgcgatgcatttgagattgttgtggaaantatggtgcgtatggtcaccaaatgagrtatacacgattcctttgtaacgataaatgtttggatgacattcaattgtagaaccactga

SEQ ID NO: 46 - DNA, 121 bp, Artificial sequence
  Marker sequence
  misc_feature (118)..(118): n is a, c, g, or t
aatcttccaaatggtctaagttatacaaccttaaagagcagccatatgattcatgtatatygactgagataaaatggaaaggtgcaagtggtggtggaaattataaacattgcaaccntca

SEQ ID NO: 47 - DNA, 121 bp, Artificial sequence
  Marker sequence
ttctattattaataaaaagaatactattatccttaaatcaacaatcttggaatcctttagygaggcaaagttaccgagtttcgtttctcttgaacttgttacaataattacaaaaccatac

SEQ ID NO: 48 - DNA, 121 bp, Artificial sequence
  Marker sequence
catttttaaatattggtaatatgcaaacatattttaagaaaatgccaagtagatgagccayagaagatacattcaatgtctccaatgtagatttatttattttttttaaaacaagagaata

SEQ ID NO: 49 - DNA, 121 bp, Artificial sequence
  Marker sequence
atgtgttgttagatctgctttctaattctcaggatcgaaagtccaatttcttgctaccttwtaaaagagctaccaacgacagcattcaagctgttaatgaagaagatgacacatcacgtcc

SEQ ID NO: 50 - DNA, 121 bp, Artificial sequence
  Marker sequence
gtctctgtataaccagcctggtgccgctggagctcctggtggggctgactcagctggacckgtgcctggttcggaaccttctggaacttcgggtggtaaggggctgaagatggtgatgtta

SEQ ID NO: 51 - DNA, 121 bp, Artificial sequence
  Marker sequence
aggagttttgggcgacgggagtgagattgccgtgaagaaagtactggaatcagatctccaygatgatgaattcaagaatgaggttgagataatcagcaagttaaggcatagaaatcttgtt

SEQ ID NO: 52 - DNA, 121 bp, Artificial sequence
  Marker sequence
  misc_feature (24)..(24): n is a, c, g, or t
agccacaacaatagaccaaaatgnatttgcttcttttgcatgacaatataaagatgatgcwtgcttcttcaaccaggcagcacaaggatgacctgttccatcgaagttatttttaccactt

SEQ ID NO: 53 - DNA, 121 bp, Artificial sequence
  Marker sequence
ttcattcaggtatttatcatctctgtggagtgctagcgcatgaccgataaagtcaattgtrttgtcatccaatccatattttgatatgagctctttagtagtcacccttgtaaggtccaat

SEQ ID NO: 54 - DNA, 121 bp, Artificial sequence
  Marker sequence
cctctgaaattaagatactttctggagtagaaacaagtgaagctgctactgtttcaggtaytggcagcgattcttcttcgtcagaactattaccttcggattcttcttctattgggttttc

SEQ ID NO: 55 - DNA, 121 bp, Artificial sequence
  Marker sequence
gaaaaagacgacgaatctgcattttcgtcctgaaagttaacgatcgccagccgcctatcaycctcagcttcttcgacgtcgccaagggaaggtgaagaatcgaactcgacgtcggagtctg

SEQ ID NO: 56 - DNA, 121 bp, Artificial sequence
  Marker sequence
  misc_feature (12)..(12): n is a, c, g, or t
tattggtaaaantaagtacaaaatataagaagattaagtttaataatcctggttcctttawattgtccagactctcccaagcaaaacaagtgagaaattagcattggcttcaaagttcaaa

SEQ ID NO: 57 - DNA, 121 bp, Artificial sequence
  Marker sequence
  misc_feature (26)..(26): n is a, c, g, or t
  misc_feature (52)..(52): n is a, c, g, or t
  misc_feature (84)..(84): n is a, c, g, or t
gattagatttcgagaatggagaaaangggagtgttggaagaaacagtaaaanggaataagygtaggtgaccgttggagattttngtttataaaatgctgatttacgattaagctttagcca

SEQ ID NO: 58 - DNA, 121 bp, Artificial sequence
  Marker sequence
tggtatacaaatacagctcgatattggttactaattgcttgatattggtatggtaataccrtaatagccctaactagctctaggtctaaaatttatcttttcatggaaaatgacatagttt

SEQ ID NO: 59 - DNA, 121 bp, Artificial sequence
  Marker sequence
agattgtgtgtttcctaggattcctcagttagcagttattggtttttcgggtagtcttgckaatctttacacgtttgagataaggtcaatgtgggtggctcattttcttgatggagggttt

SEQ ID NO: 60 - DNA, 121 bp, Artificial sequence
  Marker sequence
  misc_feature (87)..(87): n is a, c, g, or t
  misc_feature (90)..(90): n is a, c, g, or t
gccctgctccagagcttattctcacgactggacggagtgccctttcgtgcatccaggcgaraacgcgcgtcgaagagacttgaaaangtncgtctacagctgcgttccgtgtcctgagttc

SEQ ID NO: 61 - DNA, 121 bp, Artificial sequence
  Marker sequence
  misc_feature (12)..(12): n is a, c, g, or t
tattaaagtttngtccaaaagaaggcgatagtggatcaactgaatatccaacaagtccatrgttattgttgttattacgataattggatggagagcttccacctggactgccaattaaaga

SEQ ID NO: 62 - DNA, 121 bp, Artificial sequence
  Marker sequence
tgccttccagcataaacacccctgcacaaaatgctacatttgttaggacgtgtcttgctaytgagcaaaaatacccaaattggttgactcagttgcctccaaatgataataataataaaac

SEQ ID NO: 63 - DNA, 121 bp, Artificial sequence
  Marker sequence
aactgtagtacagaaataaactagtctgaacccatgcttcgcacatggaatcgcacaacaygattaaataaaatttgcatagtacatttcaggtttgcgatgtttgacaaatacatcagat

SEQ ID NO: 64 - DNA, 116 bp, Artificial sequence
  Marker sequence
  misc_feature (57)..(57): n is a, c, g, or t
  misc_feature (75)..(75): n is a, c, g, or t
ctatagtgcagagcttgaacttgaaccaaagcagtatcatgtaattgcatttgaarntccagcagattctaaaantttctgttatattgtgcaagcacatatggagatgttaggaa

SEQ ID NO: 65 - DNA, 121 bp, Artificial sequence
  Marker sequence
tcaggttggagcggacccggaaagtgcagccgcctacaatggaggtttggttaggaagttyaatggtggaggagggacgccgttgatgccgaagaggaagtttgagacgtacatttttgcg

SEQ ID NO: 66 - DNA, 121 bp, Artificial sequence
  Marker sequence
caatgagacatagccaattggcatttcgcagcactgacctaaaatggattcataatcaaayccttctaaaggcaaaccattcaaacttctattagtgattctctttacggcctcacgtcga

SEQ ID NO: 67 - DNA, 121 bp, Artificial sequence
  Marker sequence
  misc_feature (26)..(26): n is a, c, g, or t
acaattgctatcttcgtttttacatnaccgtttggtggtcgataacatagatgaatgaaaygaggaggatttgatgaagcagcagcaacacctaaatatgaacccatcttcaattccgtgc

SEQ ID NO: 68 - DNA, 235 bp, Artificial sequence
  Marker sequence
tgtggattagctactaaaaattatacatgatttcaggaaatgaagcacattattcaatcataaagcaagctcagctggttcacctggatkasgtkystgtsaarmwymmmtwmwscyrytkaaccmtmcymwmkyrrmmkkrykwtasayakgcykkkcyywykmygwrwymwttymykmkmwrscyrwwwwrmytmkkmmkmwyyaymckmmmyrttwmaykyykywrcgactc

SEQ ID NO: 69 - DNA, 121 bp, Artificial sequence
  Marker sequence
  misc_feature (97)..(97): n is a, c, g, or t
agatataactacttttggattatgggcttatgatgctgcttttgccttagcaatggctacygagtcagctcagccagcttataactatagtaatgangttgctaacggtaatttaatgaag

SEQ ID NO: 70 - DNA, 121 bp, Artificial sequence
  Marker sequence
  misc_feature (92)..(92): n is a, c, g, or t
agaaattacagttgataaagtagccgatgaaggcaatcttacactagcacaaagttttagygataaccacagtgatagggattcaagaaaancactggctcacttaacaatgagcaaatct

SEQ ID NO: 71 - DNA, 141 bp, Artificial sequence
  Marker sequence
  misc_feature (55)..(55): n is a, c, g, or t
gcattccataaccaccattcaacatgcactccactggcatgcaatatgttattanattttatgatcaagyactttcatcagctgttacaagttgtgactgttcgctgctaataacttaataattctgtcactacaacaaat

SEQ ID NO: 72 - DNA, 121 bp, Artificial sequence
  Marker sequence
  misc_feature (50)..(50): n is a, c, g, or t
  misc_feature (93)..(93): n is a, c, g, or t
tggtgtttctggagctgaagcatttggagaagtattcacattgaaggaantaggcatttgmacagtgccatagcaatttggctcagaaccagncgcacagatcaaaggatttcctacaatg

SEQ ID NO: 73 - DNA, 121 bp, Artificial sequence
  Marker sequence
tgactctatactagatgatgagttctccttctccaacctcaacttatcacatctgctattytgactaacattcattgcatcacttctgcttctttgaactctttgttgcaatccaacattc

SEQ ID NO: 74 - DNA, 121 bp, Artificial sequence
  Marker sequence
  misc_feature (11)..(11): n is a, c, g, or t
  misc_feature (24)..(24): n is a, c, g, or t
atggcttgaanggtcgctcatcancccccagcggtccgaccactctatatccaatctcctscgcctcgattatcttctcctctttactcttcccactcactttaaacttcctcacggatcc

SEQ ID NO: 75 - DNA, 20 bp, Artificial sequence
  VIC-labeled probe
agctctactcttccagcaaa

SEQ ID NO: 76 - DNA, 20 bp, Artificial sequence
  VIC-labeled probe
atgatccaatgcttttccat

SEQ ID NO: 77 - DNA, 18 bp, Artificial sequence
  VIC-labeled probe
tcacttctgataaagctt

SEQ ID NO: 78 - DNA, 17 bp, Artificial sequence
  VIC-labeled probe
ccttggagagtgttgtc

SEQ ID NO: 79 - DNA, 19 bp, Artificial sequence
  VIC-labeled probe
atcattgggaaataatcat

SEQ ID NO: 80 - DNA, 19 bp, Artificial sequence
  VIC-labeled probe
ctggtcatttgctttagct

SEQ ID NO: 81 - DNA, 18 bp, Artificial sequence
  VIC-labeled probe
atacgaaatgaaatcatc

SEQ ID NO: 82 - DNA, 19 bp, Artificial sequence
  VIC-labeled probe
ttggtcacctagaatggta

SEQ ID NO: 83 - DNA, 17 bp, Artificial sequence
  VIC-labeled probe
ctagctttgagaatcgt

SEQ ID NO: 84 - DNA, 16 bp, Artificial sequence
  VIC-labeled probe
atggactccatatttg

SEQ ID NO: 85 - DNA, 15 bp, Artificial sequence
  VIC-labeled probe
tccagcacatgcatg

SEQ ID NO: 86 - DNA, 19 bp, Artificial sequence
  VIC-labeled probe
ccacctacaataacaacac

SEQ ID NO: 87 - DNA, 19 bp, Artificial sequence
  VIC-labeled probe
actttctgttgttatcttc

SEQ ID NO: 88 - DNA, 20 bp, Artificial sequence
  VIC-labeled probe
acaattcttcatactaatcc

SEQ ID NO: 89 - DNA, 17 bp, Artificial sequence
  VIC-labeled probe
cttctcagtcgaaacag

SEQ ID NO: 90 - DNA, 19 bp, Artificial sequence
  VIC-labeled probe
ccctatagttccgattact

SEQ ID NO: 91 - DNA, 17 bp, Artificial sequence
  VIC-labeled probe
cttctcagtcgaaacag

SEQ ID NO: 92 - DNA, 15 bp, Artificial sequence
  VIC-labeled probe
ccgaaccccacaaac

SEQ ID NO: 93 - DNA, 16 bp, Artificial sequence
  VIC-labeled probe
acagccctaaattcta

SEQ ID NO: 94 - DNA, 18 bp, Artificial sequence
  VIC-labeled probe
accgctaatactaaatat

SEQ ID NO: 95 - DNA, 17 bp, Artificial sequence
  VIC-labeled probe
catcgtcatcatcatct

SEQ ID NO: 96 - DNA, 18 bp, Artificial sequence
  VIC-labeled probe
cggatgcagtaattaaga

SEQ ID NO: 97 - DNA, 21 bp, Artificial sequence
  VIC-labeled probe
tgttaatgggttttgatttag

SEQ ID NO: 98 - DNA, 20 bp, Artificial sequence
  VIC-labeled probe
agcatagaaggttataactg

SEQ ID NO: 99 - DNA, 20 bp, Artificial sequence
  VIC-labeled probe
atttcagggcaacttagaat

SEQ ID NO: 100 - DNA, 19 bp, Artificial sequence
  VIC-labeled probe
tgaagcagagtgatcagtt

SEQ ID NO: 101 - DNA, 15 bp, Artificial sequence
  VIC-labeled probe
tcgtgcaataaaagc

SEQ ID NO: 102 - DNA, 19 bp, Artificial sequence
  VIC-labeled probe
caccaaatgagatatacac

SEQ ID NO: 103 - DNA, 17 bp, Artificial sequence
  VIC-labeled probe
ctttgcctcactaaagg

SEQ ID NO: 104 - DNA, 15 bp, Artificial sequence
  VIC-labeled probe
caggcacaggtccag

SEQ ID NO: 105 - DNA, 19 bp, Artificial sequence
  VIC-labeled probe
tcagatctccatgatgatg

SEQ ID NO: 106 - DNA, 17 bp, Artificial sequence
  VIC-labeled probe
aagatgatgcatgcttc

SEQ ID NO: 107 - DNA, 17 bp, Artificial sequence
  VIC-labeled probe
tcgctgccaatacctga

SEQ ID NO: 108 - DNA, 20 bp, Artificial sequence
  VIC-labeled probe
caagaaatgagcagtaatat

SEQ ID NO: 109 - DNA, 15 bp, Artificial sequence
  VIC-labeled probe
ccgccatagctctaa

SEQ ID NO: 110 - DNA, 20 bp, Artificial sequence
  VIC-labeled probe
tgaaagtgtgtcatcaatta

SEQ ID NO: 111 - DNA, 15 bp, Artificial sequence
  VIC-labeled probe
cctggattaggcctg

SEQ ID NO: 112 - DNA, 18 bp, Artificial sequence
  VIC-labeled probe
caatggctactgagtcag

SEQ ID NO: 113 - DNA, 19 bp, Artificial sequence
  VIC-labeled probe
actgtggttatcactaaaa

SEQ ID NO: 114 - DNA, 19 bp, Artificial sequence
  VIC-labeled probe
ctgatgaaagtgcttgatc

SEQ ID NO: 115 - DNA, 16 bp, Artificial sequence
  VIC-labeled probe
gagttacctcttagct

SEQ ID NO: 116 - DNA, 18 bp, Artificial sequence
  FAM-labeled probe
ctctactcttgcagcaaa

SEQ ID NO: 117 - DNA, 19 bp, Artificial sequence
  FAM-labeled probe
tgatccaatgctcttccat

SEQ ID NO: 118 - DNA, 16 bp, Artificial sequence
  FAM-labeled probe
acttctgatgaagctt

SEQ ID NO: 119 - DNA, 15 bp, Artificial sequence
  FAM-labeled probe
ttggagagcgttgtc

SEQ ID NO: 120 - DNA, 17 bp, Artificial sequence
  FAM-labeled probe
cattgggaagtaatcat

SEQ ID NO: 121 - DNA, 18 bp, Artificial sequence
  FAM-labeled probe
tggtcatttgcgttagct

SEQ ID NO: 122 - DNA, 18 bp, Artificial sequence
  FAM-labeled probe
atacgaaatgtaatcatc

SEQ ID NO: 123 - DNA, 18 bp, Artificial sequence
  FAM-labeled probe
tggtcacctaggatggta

SEQ ID NO: 124 - DNA, 17 bp, Artificial sequence
  FAM-labeled probe
ctagctttgacaatcgt

SEQ ID NO: 125 - DNA, 16 bp, Artificial sequence
  FAM-labeled probe
atggactccgtatttg

SEQ ID NO: 126 - DNA, 13 bp, Artificial sequence
  FAM-labeled probe
cagcgcatgcatg

SEQ ID NO: 127 - DNA, 18 bp, Artificial sequence
  FAM-labeled probe
cacctacaatagcaacac

SEQ ID NO: 128 - DNA, 16 bp, Artificial sequence
  FAM-labeled probe
ttctgtcgttatcttc

SEQ ID NO: 129 - DNA, 18 bp, Artificial sequence
  FAM-labeled probe
aattcttcatgctaatcc

SEQ ID NO: 130 - DNA, 16 bp, Artificial sequence
  FAM-labeled probe
ttctcagtggaaacag

SEQ ID NO: 131 - DNA, 18 bp, Artificial sequence
  FAM-labeled probe
cctatagttcggattact

SEQ ID NO: 132 - DNA, 16 bp, Artificial sequence
  FAM-labeled probe
ttctcagtggaaacag

SEQ ID NO: 133 - DNA, 14 bp, Artificial sequence
  FAM-labeled probe
cgaaccgcacaaac

SEQ ID NO: 134 - DNA, 14 bp, Artificial sequence
  FAM-labeled probe
agccctgaattcta

SEQ ID NO: 135 - DNA, 16 bp, Artificial sequence
  FAM-labeled probe
cgctaatgctaaatat

SEQ ID NO: 136 - DNA, 17 bp, Artificial sequence
  FAM-labeled probe
catcgtcatcgtcatct

SEQ ID NO: 137 - DNA, 18 bp, Artificial sequence
  FAM-labeled probe
cggatgcagtagttaaga

SEQ ID NO: 138 - DNA, 17 bp, Artificial sequence
  FAM-labeled probe
aatgggtttcgatttag

SEQ ID NO: 139 - DNA, 18 bp, Artificial sequence
  FAM-labeled probe
catagaaggctataactg

SEQ ID NO: 140 - DNA, 17 bp, Artificial sequence
  FAM-labeled probe
tcagggcaacctagaat

SEQ ID NO: 141 - DNA, 17 bp, Artificial sequence
  FAM-labeled probe
aagcagagtggtcagtt

SEQ ID NO: 142 - DNA, 15 bp, Artificial sequence
  FAM-labeled probe
tcgtgcaatgaaagc

SEQ ID NO: 143 - DNA, 19 bp, Artificial sequence
  FAM-labeled probe
caccaaatgaggtatacac

SEQ ID NO: 144 - DNA, 16 bp, Artificial sequence
  FAM-labeled probe
tttgcctcgctaaagg

SEQ ID NO: 145 - DNA, 14 bp, Artificial sequence
  FAM-labeled probe
aggcaccggtccag

SEQ ID NO: 146 - DNA, 17 bp, Artificial sequence
  FAM-labeled probe
agatctccacgatgatg

SEQ ID NO: 147 - DNA, 18 bp, Artificial sequence
  FAM-labeled probe
aaagatgatgcttgcttc

SEQ ID NO: 148 - DNA, 16 bp, Artificial sequence
  FAM-labeled probe
cgctgccagtacctga

SEQ ID NO: 149 - DNA, 19 bp, Artificial sequence
  FAM-labeled probe
aagaaatgagcggtaatat

SEQ ID NO: 150 - DNA, 14 bp, Artificial sequence
  FAM-labeled probe
cgccatggctctaa

SEQ ID NO: 151 - DNA, 18 bp, Artificial sequence
  FAM-labeled probe
aaagtgtgtcgtcaatta

SEQ ID NO: 152 - DNA, 16 bp, Artificial sequence
  FAM-labeled probe
cctggatgacttgtgt

SEQ ID NO: 153 - DNA, 17 bp, Artificial sequence
  FAM-labeled probe
aatggctaccgagtcag

SEQ ID NO: 154 - DNA, 18 bp, Artificial sequence
  FAM-labeled probe
ctgtggttatcgctaaaa

SEQ ID NO: 155 - DNA, 19 bp, Artificial sequence
  FAM-labeled probe
ctgatgaaagtacttgatc

SEQ ID NO: 156 - DNA, 15 bp, Artificial sequence
  FAM-labeled probe
ttggagcatacccta

SEQ ID NO: 157 - DNA, 29 bp, Artificial sequence
  Taqman forward primer
tttgtaaccaaactctgaccttagatgtt

SEQ ID NO: 158 - DNA, 22 bp, Artificial sequence
  Taqman forward primer
gacgaaggtgatgatgctttgc

SEQ ID NO: 159 - DNA, 18 bp, Artificial sequence
  Taqman forward primer
cggaaggtcgcgatcctc

SEQ ID NO: 160 - DNA, 25 bp, Artificial sequence
  Taqman forward primer
ggacgatgcgatcaagactacaaat

SEQ ID NO: 161 - DNA, 24 bp, Artificial sequence
  Taqman forward primer
gtcctctagctcttttcggtgtag

SEQ ID NO: 162 - DNA, 25 bp, Artificial sequence
  Taqman forward primer
gaatcccatgatgtcaaatccgttt

SEQ ID NO: 163 - DNA, 24 bp, Artificial sequence
  Taqman forward primer
tgtgcaatttgtatccctggcata

SEQ ID NO: 164 - DNA, 25 bp, Artificial sequence
  Taqman forward primer
ctttttcctcaagctggttgtcaat

SEQ ID NO: 165 - DNA, 25 bp, Artificial sequence
  Taqman forward primer
tccatttcttcagccctactttgtc

SEQ ID NO: 166 - DNA, 17 bp, Artificial sequence
  Taqman forward primer
gagcctgcggcatcatg

SEQ ID NO: 167 - DNA, 26 bp, Artificial sequence
  Taqman forward primer
agaaatgtctgaattcagagctctgg

SEQ ID NO: 168 - DNA, 36 bp, Artificial sequence
  Taqman forward primer
attgatgtatgttgtatgtaaacaataacagtaagt

SEQ ID NO: 169 - DNA, 24 bp, Artificial sequence
  Taqman forward primer
acatttccacacgttgcattttgt

SEQ ID NO: 170 - DNA, 23 bp, Artificial sequence
  Taqman forward primer
gaacagatgggatgatgcagaga

SEQ ID NO: 171 - DNA, 20 bp, Artificial sequence
  Taqman forward primer
gggtcgctggcaattttgaa

SEQ ID NO: 172 - DNA, 20 bp, Artificial sequence
  Taqman forward primer
ctgcatcatcaccccctctt

SEQ ID NO: 173 - DNA, 22 bp, Artificial sequence
  Taqman forward primer
cttatgaccaggcagcttttgc

SEQ ID NO: 174 - DNA, 25 bp, Artificial sequence
  Taqman forward primer
cccctacctcttatcagaacatcga

SEQ ID NO: 175 - DNA, 27 bp, Artificial sequence
  Taqman forward primer
tcacagacattagtatgaaagcaagca

SEQ ID NO: 176 - DNA, 23 bp, Artificial sequence
  Taqman forward primer
ccccttcaagagcaagattctca

SEQ ID NO: 177 - DNA, 30 bp, Artificial sequence
  Taqman forward primer
gaggattcattcattcatgttaaagtgcat

SEQ ID NO: 178 - DNA, 28 bp, Artificial sequence
  Taqman forward primer
catgccccttatcttgctatttatctca

SEQ ID NO: 179 - DNA, 31 bp, Artificial sequence
  Taqman forward primer
gatattcttctctgtaaatagcctcgagatt

SEQ ID NO: 180 - DNA, 25 bp, Artificial sequence
  Taqman forward primer
ctgcaggaagcaatagaaaaagcaa

SEQ ID NO: 181 - DNA, 25 bp, Artificial sequence
  Taqman forward primer
gcttcattgtcttgctggttttcaa

SEQ ID NO: 182 - DNA, 24 bp, Artificial sequence
  Taqman forward primer
gcagagtaatcggcatgtcttctt

SEQ ID NO: 183 - DNA, 33 bp, Artificial sequence
  Taqman forward primer
cccatttgtttctaactaaatctcaaaggaaaa

SEQ ID NO: 184 - DNA, 25 bp, Artificial sequence
  Taqman forward primer
cgatgcatttgagattgttgtggaa

SEQ ID NO: 185 - DNA, 35 bp, Artificial sequence
  Taqman forward primer
taaaaagaatactattatccttaaatcaacaatct

SEQ ID NO: 186 - DNA, 17 bp, Artificial sequence
  Taqman forward primer
cgctggagctcctggtg

SEQ ID NO: 187 - DNA, 24 bp, Artificial sequence
  Taqman forward primer
attgccgtgaagaaagtactggaa

SEQ ID NO: 188 - DNA, 23 bp, Artificial sequence
  Taqman forward primer
agccacaacaatagaccaaaatg

SEQ ID NO: 189 - DNA, 25 bp, Artificial sequence
  Taqman forward primer
ggagtagaaacaagtgaagctgcta

SEQ ID NO: 190 - DNA, 25 bp, Artificial sequence
  Taqman forward primer
aggaagttgaaaaggccattaacga

SEQ ID NO: 191 - DNA, 23 bp, Artificial sequence
  Taqman forward primer
cgagtgctccctcatgtatttgg

SEQ ID NO: 192 - DNA, 25 bp, Artificial sequence
  Taqman forward primer
ccttgagtacctaggtgactatcgt

SEQ ID NO: 193 - DNA, 25 bp, Artificial sequence
  Taqman forward primer
aagagtaagaggttaaacgggttgc

SEQ ID NO: 194 - DNA, 25 bp, Artificial sequence
  Taqman forward primer
gcttatgatgctgcttttgccttag

SEQ ID NO: 195 - DNA, 25 bp, Artificial sequence
  Taqman forward primer
cgatgaaggcaatcttacactagca

SEQ ID NO: 196 - DNA, 25 bp, Artificial sequence
  Taqman forward primer
actccactggcatgcaatatgttat

SEQ ID NO: 197 - DNA, 29 bp, Artificial sequence
  Taqman forward primer
agtagaaataagtgaagaatattgatgtg

SEQ ID NO: 198 - DNA, 23 bp, Artificial sequence
  Taqman reverse primer
ggttggagatccaaattgctatc

SEQ ID NO: 199 - DNA, 24 bp, Artificial sequence
  Taqman reverse primer
gctaggctggtaggttcttttagt

SEQ ID NO: 200 - DNA, 25 bp, Artificial sequence
  Taqman reverse primer
gagctagcttggtaacaagaggatt

SEQ ID NO: 201 - DNA, 25 bp, Artificial sequence
  Taqman reverse primer
ggtaatggtattctccaaccttggt

SEQ ID NO: 202 - DNA, 26 bp, Artificial sequence
  Taqman reverse primer
cactatagtgcagtcaaagtctgagt

SEQ ID NO: 203 - DNA, 23 bp, Artificial sequence
  Taqman reverse primer
gcacttggacagcaacattttga

SEQ ID NO: 204 - DNA, 30 bp, Artificial sequence
  Taqman reverse primer
ttagattttctacctatgtcctaccaggtt

SEQ ID NO: 205 - DNA, 19 bp, Artificial sequence
  Taqman reverse primer
accttctctcaattgtgca

SEQ ID NO: 206 - DNA, 39 bp, Artificial sequence
  Taqman reverse primer
aaatcataagaattaagaattcaaaatcgaattcaaaag

SEQ ID NO: 207 - DNA, 31 bp, Artificial sequence
  Taqman reverse primer
tttaccaaagtaattctaaataaggattgtt

SEQ ID NO: 208 - DNA, 21 bp, Artificial sequence
  Taqman reverse primer
gagtcccgattgttggcaaac

SEQ ID NO: 209 - DNA, 24 bp, Artificial sequence
  Taqman reverse primer
caaagcaactcccagttcttcaac

SEQ ID NO: 210 - DNA, 30 bp, Artificial sequence
  Taqman reverse primer
ttttaccaaaagcacttttatattattgtt

SEQ ID NO: 211 - DNA, 25 bp, Artificial sequence
  Taqman reverse primer
ctctatacaactccatccaggcaat

SEQ ID NO: 212 - DNA, 25 bp, Artificial sequence
  Taqman reverse primer
gcttttaggcacttgacttctctca

SEQ ID NO: 213 - DNA, 23 bp, Artificial sequence
  Taqman reverse primer
cggaaattgtacggcgggaatat

SEQ ID NO: 214 - DNA, 25 bp, Artificial sequence
  Taqman reverse primer
gcttttaggcacttgacttctctca

SEQ ID NO: 215 - DNA, 25 bp, Artificial sequence
  Taqman reverse primer
ggcaatttttgatgaggcaatggaa

SEQ ID NO: 216 - DNA, 28 bp, Artificial sequence
  Taqman reverse primer
gcaagatgcaaaactcaaatttctagca

SEQ ID NO: 217 - DNA, 24 bp, Artificial sequence
  Taqman reverse primer
gccctgatcttgagtgtagtttgg

SEQ ID NO: 218 - DNA, 25 bp, Artificial sequence
  Taqman reverse primer
gcaagggtaagaaaatcgaaaacca

SEQ ID NO: 219 - DNA, 25 bp, Artificial sequence
  Taqman reverse primer
cagttaagaagggattcctctgcat

SEQ ID NO: 220 - DNA, 24 bp, Artificial sequence
  Taqman reverse primer
tgggtcctactttgtttgttggat

SEQ ID NO: 221 - DNA, 35 bp, Artificial sequence
  Taqman reverse primer
aacataattaataaataagtgtaactttgcatgaa

SEQ ID NO: 222 - DNA, 25 bp, Artificial sequence
  Taqman reverse primer
cctgccttttcacatttttcccatt

SEQ ID NO: 223 - DNA, 20 bp, Artificial sequence
  Taqman reverse primer
gtcgtactctcctgcaccaa

SEQ ID NO: 224 - DNA, 27 bp, Artificial sequence
  Taqman reverse primer
tgattgactgattgtgtagcttgaaga

SEQ ID NO: 225 - DNA, 30 bp, Artificial sequence
  Taqman reverse primer
gtcatccaaacatttatcgttacaaaggaa

SEQ ID NO: 226 - DNA, 26 bp, Artificial sequence
  Taqman reverse primer
agttcaagagaaacgaaactcggtaa

SEQ ID NO: 227 - DNA, 21 bp, Artificial sequence
  Taqman reverse primer
cacccgaagttccagaaggtt

SEQ ID NO: 228 - DNA, 27 bp, Artificial sequence
  Taqman reverse primer
gccttaacttgctgattatctcaacct

SEQ ID NO: 229 - DNA, 19 bp, Artificial sequence
  Taqman reverse primer
ccttgtgctgcctggttga

SEQ ID NO: 230 - DNA, 26 bp, Artificial sequence
  Taqman reverse primer
tccgaaggtaatagttctgacgaaga

SEQ ID NO: 231 - DNA, 29 bp, Artificial sequence
  Taqman reverse primer
ctttttgaaccatttcttttctcctgtct

SEQ ID NO: 232 - DNA, 25 bp, Artificial sequence
  Taqman reverse primer
cctaccaaaacgccaaagaattaca

SEQ ID NO: 233 - DNA, 33 bp, Artificial sequence
  Taqman reverse primer
tcttgaatctctctgttaatagttcaaatcgtg

SEQ ID NO: 234 - DNA, 30 bp, Artificial sequence
  Taqman reverse primer
aattatacatgatttcaggaaatgaagcac

SEQ ID NO: 235 - DNA, 28 bp, Artificial sequence
  Taqman reverse primer
tcattactatagttataagctggctgag

SEQ ID NO: 236 - DNA, 23 bp, Artificial sequence
  Taqman reverse primer
gctcattgttaagtgagccagtg

SEQ ID NO: 237 - DNA, 24 bp, Artificial sequence
  Taqman reverse primer
agcgaacagtcacaacttgtaaca

SEQ ID NO: 238 - DNA, 24 bp, Artificial sequence
  Taqman reverse primer
tggtttgagcttgttggtttggag

SEQ ID NO: 239 - DNA, 28 bp, Artificial sequence
  Taqman forward primer
atcattttagccatatcgtaaattgtca

SEQ ID NO: 240 - DNA, 25 bp, Artificial sequence
  Taqman forward primer
tacaatatgatacagaaaatcagag